European Patent Application EP 4 751 731 A1, published June 3, 2026. Title: Combination of a bispecific antibody construct, an immune checkpoint inhibitor and a taxane. Applicant: Affimed GmbH. Application EP. The sequence listing filed with the application follows.

SEQUENCE LISTING (73 sequences)

SEQ ID NO: 1 - protein, 6 aa, Synthetic construct
GGSGGS

SEQ ID NO: 2 - protein, 18 aa, Synthetic construct
GGSGGSGGSGGSGGSGGS

SEQ ID NO: 3 - protein, 21 aa, Synthetic construct
GGSGGSGGSGGSGGSGGSGGS

SEQ ID NO: 4 - protein, 9 aa, Synthetic construct
GGSGGSGGS

SEQ ID NO: 5 - protein, 5 aa, Synthetic construct
GGGGS

SEQ ID NO: 6 - protein, 10 aa, Synthetic construct
GGGGSGGGGS

SEQ ID NO: 7 - protein, 20 aa, Synthetic construct
GGGGSGGGGSGGGGSGGGGS

SEQ ID NO: 8 - protein, 30 aa, Synthetic construct
GGGGSGGGGSGGGGSGGGGSGGGGSGGGGS

SEQ ID NO: 9 - protein, 8 aa, Synthetic construct
GYTFTSYY

SEQ ID NO: 10 - protein, 8 aa, Synthetic construct
INPSGGST

SEQ ID NO: 11 - protein, 13 aa, Synthetic construct
ARGSAYYYDFADY

SEQ ID NO: 12 - protein, 6 aa, Synthetic construct
NIGSKN

SEQ ID NO: 13 - protein, 9 aa, Synthetic construct
QVWDNYSVL

SEQ ID NO: 14 - protein, 120 aa, Synthetic construct
QVQLVQSGAEVKKPGESLKVSCKASGYTFTSYYMHWVRQAPGQGLEWMGIINPSGGSTSYAQKFQGRVTMTRDTSTSTVYMELSSLRSEDTAVYYCARGSAYYYDFADYWGQGTLVTVSS

SEQ ID NO: 15 - protein, 106 aa, Synthetic construct
SYVLTQPSSVSVAPGQTATISCGGHNIGSKNVHWYQQRPGQSPVLVIYQDNKRPSGIPERFSGSNSGNTATLTISGTQAMDEADYYCQVWDNYSVLFGGGTKLTVL

SEQ ID NO: 16 - protein, 255 aa, Synthetic construct
QVQLVQSGAEVKKPGESLKVSCKASGYTFTSYYMHWVRQAPGQGLEWMGIINPSGGSTSYAQKFQGRVTMTRDTSTSTVYMELSSLRSEDTAVYYCARGSAYYYDFADYWGQGTLVTVSSGGSGGSGGSGGSGGSGGSSYVLTQPSSVSVAPGQTATISCGGHNIGSKNVHWYQQRPGQSPVLVIYQDNKRPSGIPERFSGSNSGNTATLTISGTQAMDEADYYCQVWDNYSVLFGGGTKLTVLAAAGSHHHHHH

SEQ ID NO: 17 - protein, 8 aa, Synthetic construct
GYTFTSYY

SEQ ID NO: 18 - protein, 8 aa, Synthetic construct
IEPMYGST

SEQ ID NO: 19 - protein, 13 aa, Synthetic construct
ARGSAYYYDFADY

SEQ ID NO: 20 - protein, 6 aa, Synthetic construct
NIGSKN

SEQ ID NO: 21 - protein, 9 aa, Synthetic construct
QVWDNYSVL

SEQ ID NO: 22 - protein, 120 aa, Synthetic construct
QVQLVQSGAEVKKPGESLKVSCKASGYTFTSYYMHWVRQAPGQGLEWMGAIEPMYGSTSYAQKFQGRVTMTRDTSTSTVYMELSSLRSEDTAVYYCARGSAYYYDFADYWGQGTLVTVSS

SEQ ID NO: 23 - protein, 106 aa, Synthetic construct; identical to SEQ ID NO: 15

SEQ ID NO: 24 - protein, 255 aa, Synthetic construct
QVQLVQSGAEVKKPGESLKVSCKASGYTFTSYYMHWVRQAPGQGLEWMGAIEPMYGSTSYAQKFQGRVTMTRDTSTSTVYMELSSLRSEDTAVYYCARGSAYYYDFADYWGQGTLVTVSSGGSGGSGGSGGSGGSGGSSYVLTQPSSVSVAPGQTATISCGGHNIGSKNVHWYQQRPGQSPVLVIYQDNKRPSGIPERFSGSNSGNTATLTISGTQAMDEADYYCQVWDNYSVLFGGGTKLTVLAAAGSHHHHHH

SEQ ID NO: 25 - protein, 8 aa, Synthetic construct
GYTFTNYY

SEQ ID NO: 26 - protein, 8 aa, Synthetic construct
INPSGGVT

SEQ ID NO: 27 - protein, 13 aa, Synthetic construct
ARGSAYYYDFADY

SEQ ID NO: 28 - protein, 6 aa, Synthetic construct
NIGSKS

SEQ ID NO: 29 - protein, 9 aa, Synthetic construct
QVWDDYIVL

SEQ ID NO: 30 - protein, 120 aa, Synthetic construct
QVQLVQSGAEVKKPGESLKVSCKASGYTFTNYYMQWVRQAPGQGLEWMGIINPSGGVTSYAQKFQGRVTMTRDTSTSTVYMELSSLRSEDTAVYYCARGSAYYYDFADYWGQGTLVTVSS

SEQ ID NO: 31 - protein, 106 aa, Synthetic construct
SYVLTQPSSVSVAPGQTARITCGGNNIGSKSVHWYQQKPGQAPVLVIYQDKKRPSGIPERFSGSNSGNTATLTISGTQAMDEADYYCQVWDDYIVLFGGGTKLTVL

SEQ ID NO: 32 - protein, 5 aa, Synthetic construct
SYYMH

SEQ ID NO: 33 - protein, 17 aa, Synthetic construct
AIEPRYGSTSYAQKFQG

SEQ ID NO: 34 - protein, 11 aa, Synthetic construct
GSAYYYDFADY

SEQ ID NO: 35 - protein, 11 aa, Synthetic construct
GGHNIGSKNVH

SEQ ID NO: 36 - protein, 7 aa, Synthetic construct
QDNKRPS

SEQ ID NO: 37 - protein, 9 aa, Synthetic construct
QVWDNYNVL

SEQ ID NO: 38 - protein, 5 aa, Synthetic construct
NYYMQ

SEQ ID NO: 39 - protein, 17 aa, Synthetic construct
IINPSGGVTSYAQKFQG

SEQ ID NO: 40 - protein, 11 aa, Synthetic construct
GSAYYYDFADY

SEQ ID NO: 41 - protein, 11 aa, Synthetic construct
GGNNIGSKSVH

SEQ ID NO: 42 - protein, 7 aa, Synthetic construct
QDKKRPS

SEQ ID NO: 43 - protein, 9 aa, Synthetic construct
QVWDDYIVL

SEQ ID NO: 44 - protein, 120 aa, Synthetic construct
EVQLVQSGAEVKKPGASVKVSCKASGYTFTSYYMHWVRQAPGQCLEWMGAIEPTYGSTSYAQKFQGRVTMTRDTSTSTVYMELSSLRSEDTAVYYCARGSAYYYDFADYWGQGTLVTVSS

SEQ ID NO: 45 - protein, 106 aa, Synthetic construct
SYELTQPLSVSVALGQTARITCGGHNIGSKNVHWYQQKPGQAPVLVIYQDNKRPSGIPERFSGSNSGNTATLTISRAQAGDEADYYCQVWDNYNVLFGCGTKLTVL

SEQ ID NO: 46 - protein, 120 aa, Synthetic construct
QVQLVQSGAEVKKPGASVKVSCKASGYTFTSYYMHWVRQAPGQCLEWMGAIEPTYGSTSYAQKFQGRVTMTRDTSTSTVYMELSSLRSEDTAVYYCARGSAYYYDFADYWGQGTLVTVSS

SEQ ID NO: 47 - protein, 106 aa, Synthetic construct; identical to SEQ ID NO: 45

SEQ ID NO: 48 - protein, 120 aa, Synthetic construct
QVQLVQSGAEVKKPGASVKVSCKASGYTFTSYYMHWVRQAPGQCLEWMGAIEPRYGSTSYAQKFQGRVTMTRDTSTSTVYMELSSLRSEDTAVYYCARGSAYYYDFADYWGQGTLVTVSS

SEQ ID NO: 49 - protein, 106 aa, Synthetic construct; identical to SEQ ID NO: 45

SEQ ID NO: 50 - protein, 119 aa, Synthetic construct
QVQLVQSGAEVKKPGASVKVSCKASGYTFTSYYMHWVRQAPGQCLEWMGAIEPTYGSTSYAQKFQGRVTMTRDTSTSTVYMELSSLRSEDTAVYYCARGSAYYYDFADYWGQGTLVTVS

SEQ ID NO: 51 - protein, 106 aa, Synthetic construct; identical to SEQ ID NO: 45

SEQ ID NO: 52 - protein, 120 aa, Synthetic construct
QVQLVQSGAEVKKPGASVKVSCKASGYTFTNYYMQWVRQAPGQCLEWMGIINPSGGVTSYAQKFQGRVTMTRDTSTSTVYMELSSLRSEDTAVYYCARGSAYYYDFADYWGQGTLVTVSS

SEQ ID NO: 53 - protein, 106 aa, Synthetic construct
SYELTQPLSVSVALGQTARITCGGNNIGSKSVHWYQQKPGQAPVLVIYQDKKRPSGIPERFSGSNSGNTATLTISRAQAGDEADYYCQVWDDYIVLFGCGTKLTVL

SEQ ID NO: 54 - protein, 121 aa, Synthetic construct
QVQLVQSGAEVKKPGASVKVSCKASGYTFTNYYMQWVRQAPGQCLEWMGIINPSGGVTSYAQKFQGRVTMTRDTSTSTVYMELSSLRSEDTAVYYCARGSAYYYDFADYWGQGTLVTVSSG

SEQ ID NO: 55 - protein, 106 aa, Synthetic construct; identical to SEQ ID NO: 53

SEQ ID NO: 56 - protein, 10 aa, Synthetic construct
GGSVSSGSYY

SEQ ID NO: 57 - protein, 7 aa, Synthetic construct
IYYSGST

SEQ ID NO: 58 - protein, 12 aa, Synthetic construct
ARNPISIPAFDI

SEQ ID NO: 59 - protein, 6 aa, Synthetic construct
NIGSKS

SEQ ID NO: 60 - protein, 11 aa, Synthetic construct
QVWDTSSDHVL

SEQ ID NO: 61 - protein, 120 aa, Synthetic construct
QVQLQESGPGLVKPSETLSLTCTVSGGSVSSGSYYWSWIRQPPGKGLEWIGYIYYSGSTNYNPSLKSRVTISVDTSKNQFSLKLSSVTAADTAVYYCARNPISIPAFDIWGQGTMVTVSS

SEQ ID NO: 62 - protein, 108 aa, Synthetic construct
QPVLTQPPSVSVAPGKTARITCGGNNIGSKSVHWYQQKPGQAPVLVIYYDSDRPSGIPERFSGSNSGNTATLTISRVEAGDEADYYCQVWDTSSDHVLFGGGTKLTVL

SEQ ID NO: 63 - protein, 705 aa, Synthetic construct
QVQLVQSGAEVKKPGESLKVSCKASGYTFTSYYMHWVRQAPGQGLEWMGIINPSGGSTSYAQKFQGRVTMTRDTSTSTVYMELSSLRSEDTAVYYCARGSAYYYDFADYWGQGTLVTVSSASTKGPSVFPLAPSSKSTSGGTAALGCLVKDYFPEPVTVSWNSGALTSGVHTFPAVLQSSGLYSLSSVVTVPSSSLGTQTYICNVNHKPSNTKVDKKVEPKSCDKTHTCPPCPAPEFEGGPSVFLFPPKPKDTLMISRTPEVTCVVVAVSHEDPEVKFNWYVDGVEVHNAKTKPREEQYNSTYRVVSVLTVLHQDWLNGKEYKCKVSNKALPAPIEKTISKAKGQPREPQVYTLPPSREEMTKNQVSLTCLVKGFYPSDIAVEWESNGQPENNYKTTPPVLDSDGSFFLYSKLTVDKSRWQQGNVFSCSVMHEALHNHYTQKSLSLSPGGGGGSGGGGSQVQLQESGPGLVKPSETLSLTCTVSGGSVSSGSYYWSWIRQPPGKGLEWIGYIYYSGSTNYNPSLKSRVTISVDTSKNQFSLKLSSVTAADTAVYYCARNPISIPAFDIWGQGTMVTVSSGGSGGSGGSGGSGGSGGSQPVLTQPPSVSVAPGKTARITCGGNNIGSKSVHWYQQKPGQAPVLVIYYDSDRPSGIPERFSGSNSGNTATLTISRVEAGDEADYYCQVWDTSSDHVLFGGGTKLTVL

SEQ ID NO: 64 - protein, 212 aa, Synthetic construct
SYVLTQPSSVSVAPGQTATISCGGHNIGSKNVHWYQQRPGQSPVLVIYQDNKRPSGIPERFSGSNSGNTATLTISGTQAMDEADYYCQVWDNYSVLFGGGTKLTVLGQPKAAPSVTLFPPSSEELQANKATLVCLISDFYPGAVTVAWKADSSPVKAGVETTTPSKQSNNKYAASSYLSLTPEQWKSHRSYSCQVTHEGSTVEKTVAPTECS

SEQ ID NO: 65 - protein, 705 aa, Synthetic construct
QVQLVQSGAEVKKPGESLKVSCKASGYTFTSYYMHWVRQAPGQGLEWMGAIEPMYGSTSYAQKFQGRVTMTRDTSTSTVYMELSSLRSEDTAVYYCARGSAYYYDFADYWGQGTLVTVSSASTKGPSVFPLAPSSKSTSGGTAALGCLVKDYFPEPVTVSWNSGALTSGVHTFPAVLQSSGLYSLSSVVTVPSSSLGTQTYICNVNHKPSNTKVDKKVEPKSCDKTHTCPPCPAPEFEGGPSVFLFPPKPKDTLMISRTPEVTCVVVAVSHEDPEVKFNWYVDGVEVHNAKTKPREEQYNSTYRVVSVLTVLHQDWLNGKEYKCKVSNKALPAPIEKTISKAKGQPREPQVYTLPPSREEMTKNQVSLTCLVKGFYPSDIAVEWESNGQPENNYKTTPPVLDSDGSFFLYSKLTVDKSRWQQGNVFSCSVMHEALHNHYTQKSLSLSPGGGGGSGGGGSQVQLQESGPGLVKPSETLSLTCTVSGGSVSSGSYYWSWIRQPPGKGLEWIGYIYYSGSTNYNPSLKSRVTISVDTSKNQFSLKLSSVTAADTAVYYCARNPISIPAFDIWGQGTMVTVSSGGSGGSGGSGGSGGSGGSQPVLTQPPSVSVAPGKTARITCGGNNIGSKSVHWYQQKPGQAPVLVIYYDSDRPSGIPERFSGSNSGNTATLTISRVEAGDEADYYCQVWDTSSDHVLFGGGTKLTVL

SEQ ID NO: 66 - protein, 212 aa, Synthetic construct; identical to SEQ ID NO: 64

SEQ ID NO: 67 - protein, 489 aa, Synthetic construct
QVQLQESGPGLVKPSETLSLTCTVSGGSVSSGSYYWSWIRQPPGKGLEWIGYIYYSGSTNYNPSLKSRVTISVDTSKNQFSLKLSSVTAADTAVYYCARNPISIPAFDIWGQGTMVTVSSGGSGGSGGSSYVLTQPSSVSVAPGQTATISCGGHNIGSKNVHWYQQRPGQSPVLVIYQDNKRPSGIPERFSGSNSGNTATLTISGTQAMDEADYYCQVWDNYSVLFGGGTKLTVLGGSGGSQVQLVQSGAEVKKPGESLKVSCKASGYTFTSYYMHWVRQAPGQGLEWMGIINPSGGSTSYAQKFQGRVTMTRDTSTSTVYMELSSLRSEDTAVYYCARGSAYYYDFADYWGQGTLVTVSSGGSGGSGGSQPVLTQPPSVSVAPGKTARITCGGNNIGSKSVHWYQQKPGQAPVLVIYYDSDRPSGIPERFSGSNSGNTATLTISRVEAGDEADYYCQVWDTSSDHVLFGGGTKLTVLAAAGSHHHHHH

SEQ ID NO: 68 - protein, 505 aa, Synthetic construct
SYVLTQPSSVSVAPGQTATISCGGHNIGSKNVHWYQQRPGQSPVLVIYQDNKRPSGIPERFSGSNSGNTATLTISGTQAMDEADYYCQVWDNYSVLFGGGTKLTVLGQPKAAPSVTLFPPSSEELQANKATLVCLISDFYPGAVTVAWKADSSPVKAGVETTTPSKQSNNKYAASSYLSLTPEQWKSHRSYSCQVTHEGSTVEKTVAPTECSLTVDKSRWQQGNVFSCSVMHEALHNHYTQKSLSLSPGGGGGSGGGGSQVQLQESGPGLVKPSETLSLTCTVSGGSVSSGSYYWSWIRQPPGKGLEWIGYIYYSGSTNYNPSLKSRVTISVDTSKNQFSLKLSSVTAADTAVYYCARNPISIPAFDIWGQGTMVTVSSGGSGGSGGSGGSGGSGGSQPVLTQPPSVSVAPGKTARITCGGNNIGSKSVHWYQQKPGQAPVLVIYYDSDRPSGIPERFSGSNSGNTATLTISRVEAGDEADYYCQVWDTSSDHVLFGGGTKLTVL

SEQ ID NO: 69 - protein, 231 aa, Synthetic construct
EPKSCDKTHTCPPCPAPEFEGGPSVFLFPPKPKDTLMISRTPEVTCVVVAVSHEDPEVKFNWYVDGVEVHNAKTKPREEQYNSTYRVVSVLTVLHQDWLNGKEYKCKVSNKALPAPIEKTISKAKGQPREPQVYTLPPSREEMTKNQVSLTCLVKGFYPSDIAVEWESNGQPENNYKTTPPVLDSDGSFFLYSKLTVDKSRWQQGNVFSCSVMHEALHNHYTQKSLSLSPG

SEQ ID NO: 70 - protein, 8 aa, Synthetic construct
SFFPPGYQ

SEQ ID NO: 71 - protein, 254 aa, Homo sapiens
MWQLLLPTALLLLVSAGMRTEDLPKAVVFLEPQWYRVLEKDSVTLKCQGAYSPEDNSTQWFHNESLISSQASSYFIDAATVDDSGEYRCQTNLSTLSDPVQLEVHIGWLLLQAPRWVFKEEDPIHLRCHSWKNTALHKVTYLQNGKGRKYFHHNSDFYIPKATLKDSGSYFCRGLFGSKNVSSETVNITITQGLAVSTISSFFPPGYQVSFCLVMVLLFAVDTGLYFSVKTNIRSSTRDWKDHKFKWRKDPQDK

SEQ ID NO: 72 - protein, 4 aa, Synthetic construct
GGGS

SEQ ID NO: 73 - protein, 6 aa, Synthetic construct
HHHHHH